European Patent Specification EP 3 231 446 B1, published January 7, 2026. Title: COMPOSITIONS AND METHODS FOR SELECTIVE DELIVERY OF OLIGONUCLEOTIDE MOLECULES TO SPECIFIC NEURON TYPES. Applicant: nLife Therapeutics S.L. The sequence listing filed with the application follows.

SEQUENCE LISTING (70 sequences)

SEQ ID NO: 1 - RNA, 70 nt, Mus musculus
ggugguaguggugguaauagugguggugauggagaaggaagaaguggaggaagaguguagggcuuacagg

SEQ ID NO: 2 - RNA, 110 nt, Mus musculus
caacaccacaacgucccuggagcccuucgggacaggcggcaacgauacuggccucuccaacgugaccuucagcuaccaagugaucaccucucuuuugcuggggacgcuca

SEQ ID NO: 3 - RNA, 110 nt, Mus musculus
gcccauggcugcucuguaccaggugcucaacaaguggacucugggucaggucaccugugaccuguuuaucgcccuggaugugcugugcugcacuucguccauccugcacc

SEQ ID NO: 4 - RNA, 2321 nt, Mus musculus
ugauaguugcaauaaccuccucucuauucgaaaucccaauucuucacgauggaaguuuaaaccucggcgauucaaggaagaaaacccaaacagaaaauauaaacuguauggacaucuaccaugcccacuaggacugccacccucugcccuauaucuggaacuuugagguucaagacugcucugucucucccucccucuugcucuagaaacaucuguucccuuugggugucaauguacacugcugauucuggucuccaugcacucacggcuggucugggaaaguuggaacuacuuuggguuauggugcccuggaauuguuugccuugcugaauagcaaaagaucccuuuccccaaugcacagcacccacuuucuguauuuuguuuguuuguuuguuuuaacucaaaaucaagugacaaagaugucugcuggaguggacuuauaagcaagaagccaggcccaaaaggaagagccaagaaggccugcggauguuuuccuguccuggugucagcacucaccaaagaaauugacaaucagacuauuuggaaggaagaguuuuauuccuguaguuuguuggcuuuucuguaaguucuggaaaggccuuguggacugcagaaggcgcccacugcuggccagggagggcucauugagggugcugagaugcccgggauggcucaccucacccucaguuucuuuucuaggagugagcuaugccagagcagcucaccuugaguuugcagccuccggguuccuccacucaccucucacaguauccaggagcuaguagagaaguuugaguuugugcaagagguuggagacuuagaauuucuaaggaagugugggugugaggcacguagaggagguaaggagcaaaagggcuccuaagugcuuccaacuccugcggcgugcccagggggugggggugaccuaaaggggcaauuuuaagcauaggaugcaaaguuucucaaucuaccccuucccccuuucaaggaacagcauuguguagcauuuccuaaaaaugcccggauuuauucuccgggacauucugugcucacacaaauuucgcagaucucugggcucucauugugaaggguaucaacaccucaccauuaccuaccuaggaucuugaucucagagaccuaaaagagagagcgaucucuguggagucccagccaagucagcccccaaauucugaggguaaaaccaguuuuguguccucucaauuuuuaaagcauuuuucuccgcuagggguucuuuuccugcuguuauuuuugcugucccacccccaccucagagaagaaaauuauuuaggugcuuccuuugaauguacauuucuagcuaagugagagggcaucaaaugguuuugcguuauaucugaacuucgaauuuucuguugaauaaugguuuccuuuucaagcaauuauacggagauuuuuuucaccccccauccccuucagcuguaucuuuccaaugucugcaccugcuguuuugaaaacccgugcugcauuuuuuuuuaaauugccaaaguugcuggugagaucucccccuuguguuuauaaacagggagaaaggacugcccugccacaugaagccauuguuuuuauuuguuaaacugagcaaaguuucuuuugcucuacucuaaagugggaaugaguauuacagucccuugcaacagagccauuucagaauguaagccuguaggguguccacaccugagagacugacaggggguucuguggagaagacgcacugggcugggcuucuccaguacaaacaguacuuguuuguaaauuuagcuugcuuuauuuguuuguuuguuuauuuauuuaucacaaaaaugaaguagaacuauauggccaaauaauauuuuucuguaugcuuuacuauuuuuagaccagaucauuuacuugaaauaaagaucauuuacuugaaauaaaucaaucccuaaauuucagauguuaaauuggaaaccaagaccucuaacuuccaguucucuguauuuuuuuuuuuccaauuaggaauguuugaccgugaugggggaggggcauugcucuuguuacuuugagaaagagacuuuaaacaagacuggaaagggggcacccagcuggaauauaauugccaaguaauagagcaaucagagaacuaagugcaacaugccgcacagcucuaaagaaccccugaugcuuguuuuauuuuaaaauacuuguauuacaguaaaauguuaaugcaucaaaauuggccuucacuuuuccuugugauaauaaaggacuuuaguaauggcaaugcuguaauaaacuaagaccaguaaccuauauguaccuuu

SEQ ID NO: 5 - RNA, 19 nt, Artificial
  Sense strand of mouse 5-HT1A-specific siRNA
ggaagaguguagggcuuac

SEQ ID NO: 6 - RNA, 19 nt, Artificial
  Antisense strand of mouse 5-HT1A-specific siRNA
guaagcccuacacucuucc

SEQ ID NO: 7 - RNA, 19 nt, Artificial
  Sense strand of a mouse 5-HT1A-specific siRNA
cgauacuggccucuccaac

SEQ ID NO: 8 - RNA, 19 nt, Artificial
  Antisense strand of a mouse 5-HT1A-specific siRNA
guuggagaggccaguaucg

SEQ ID NO: 9 - RNA, 19 nt, Artificial
  Sense strand of a mouse 5-HT1A-specific siRNA
ggugcucaacaaguggacu

SEQ ID NO: 10 - RNA, 19 nt, Artificial
  Antisense strand of a mouse 5-HT1A-specific siRNA
aguccacuuguugagcacc

SEQ ID NO: 11 - RNA, 19 nt, Artificial
  Sense strand of a mouse 5-HT1A-specific siRNA
cgauggaaguuuaaaccuc

SEQ ID NO: 12 - RNA, 19 nt, Artificial
  Antisense strand of a mouse 5-HT1A-specific siRNA
gagguuuaaacuuccaucg

SEQ ID NO: 13 - DNA, 21 bp, Artificial
  Sense strand of a SERT-specific siRNA
cuccuggaacacuggcaactt

SEQ ID NO: 14 - DNA, 21 bp, Artificial
  Sense strand synucleic-specific siRNA
gcuagcuacaacaaguucatt

SEQ ID NO: 15 - DNA, 21 bp, Artificial
  Antisense strand SERT-specific siRNA
ugaacuuguuguagcuagctt

SEQ ID NO: 16 - DNA, 20 bp, Artificial
  alpha-synuclein siRNA
ggaaagacaaaagaggugtt

SEQ ID NO: 17 - DNA, 20 bp, Artificial
  alpha-synuclein siRNA
ggaaagacaaaagaggugtt

SEQ ID NO: 18 - DNA, 21 bp, Artificial
  alpha-synuclein siRNA
ggaggaauuuuagaagaggtt

SEQ ID NO: 19 - DNA, 21 bp, Artificial
  alpha-synucleic siRNA
uguuggaggagcaguggugtt

SEQ ID NO: 20 - DNA, 21 bp, Artificial
  GGACCAGUUGGGCAAGAAUTT
ggaccaguugggcaagaautt

SEQ ID NO: 21 - DNA, 63 bp, Artificial
  alpha-synuclein hairpins antisense
gatccccggaccagttgggcaagaatttcaagagaattcttgccaactggtcctttttggaaa

SEQ ID NO: 22 - DNA, 64 bp, Artificial
  alpha-synuclein hairpin antisense
ctagtttccaaaaaggaccagttgggcaagaattctcttgaaattcttgcccaactggtccggg

SEQ ID NO: 23 - DNA, 21 bp, Artificial
  synuclein siRNA
gguguggcaacaguggcugag

SEQ ID NO: 24 - DNA, 21 bp, Artificial
  Synuclein siRNA
aacaguggcugagaagaccaa

SEQ ID NO: 25 - DNA, 21 bp, Artificial
  Synuclein siRNA
auugcagcagccacuggcuuu

SEQ ID NO: 26 - DNA, 21 bp, Artificial
  Synuclein siRNA
aagugacaaauguuggaggag

SEQ ID NO: 27 - DNA, 21 bp, Artificial
  Synuclein siRNA
gaagaaggagccccacaggaa

SEQ ID NO: 28 - DNA, 21 bp, Artificial
  Synuclein siRNA
cgggugugacagcaguagctt

SEQ ID NO: 29 - DNA, 21 bp, Artificial
  Synuclein siRNA
uccugacaaugaggcuuautt

SEQ ID NO: 30 - DNA, 21 bp, Artificial
  Synuclein SiRNA
uccugacaaugaggcuuautt

SEQ ID NO: 31 - DNA, 21 bp, Artificial
  Synuclein siRNA
cuacgaaccugaagccuaatt

SEQ ID NO: 32 - DNA, 21 bp, Artificial
  Synuclein siRNA
cuacgaaccugaagccuaatt

SEQ ID NO: 33 - DNA, 21 bp, Artificial
  Synuclein siRNA
cuacgaaccugaagccuaatt

SEQ ID NO: 34 - DNA, 21 bp, Artificial
  Synuclein siRNA
cuauuguagaguggucuautt

SEQ ID NO: 35 - DNA, 20 bp, Artificial
  Synuclein siRNA
cuaugagccugaagcuaatt

SEQ ID NO: 36 - DNA, 21 bp, Artificial
  Synuclein siRNA
cuaugagccugaagccuaatt

SEQ ID NO: 37 - DNA, 23 bp, Artificial
  dopamine beta-hydroxylase siRNA
gaccacguacuggugcuacauta

SEQ ID NO: 38 - DNA, 21 bp, Artificial
  BAX siRNA
ucgauccuggaugaaaccctg

SEQ ID NO: 39 - DNA, 21 bp, Artificial
  tau siRNA
aatcacacccaacgtgcagaa

SEQ ID NO: 40 - DNA, 21 bp, Artificial
  tau siRNA
aactggcagttctggagcaaa

SEQ ID NO: 41 - DNA, 22 bp, Artificial
  tau siRNA (sense)
tcgaagtgatggaagatcacgc

SEQ ID NO: 42 - DNA, 22 bp, Artificial
  tau siRNA (antisense)
cttcactaccttctagtgcgac

SEQ ID NO: 43 - DNA, 22 bp, Artificial
  tau siRNA (sense)
cagccgggagtcggcaaggtgc

SEQ ID NO: 44 - DNA, 22 bp, Artificial
  tau siRNA (antisense)
cggccctcagcccttccacgtc

SEQ ID NO: 45 - DNA, 24 bp, Artificial
  tau siRNA (sense)
acgtcctcggcggcggcagtgtgc

SEQ ID NO: 46 - DNA, 24 bp, Artificial
  tau SiRNA (antisense)
caggcgcctgcggcgtcacacgtt

SEQ ID NO: 47 - DNA, 21 bp, Artificial
  tau siRNA (sense)
acgtctccatggcatctcagc

SEQ ID NO: 48 - DNA, 21 bp, Artificial
  tau siRNA antisense
ttgctgagatgccatggagac

SEQ ID NO: 49 - DNA, 22 bp, Artificial
  tau siRNA (sense)
gtggccagatggaagtaaaatc

SEQ ID NO: 50 - DNA, 22 bp, Artificial
  tau siRNA (antisense)
ccggtctaccttcattttagac

SEQ ID NO: 51 - DNA, 22 bp, Artificial
  tau siRNA (sense)
gtggccagatgcaagtaaaatc

SEQ ID NO: 52 - DNA, 22 bp, Artificial
  tau siRNA (antisense)
ccggtctacgttcattttagac

SEQ ID NO: 53 - DNA, 25 bp, Artificial
  tau siRNA
ggttcagccatgctgcttcaaagcc

SEQ ID NO: 54 - DNA, 25 bp, Artificial
  tau siRNA
tgataatcgacaggaggcgaggaca

SEQ ID NO: 55 - DNA, 21 bp, Artificial
  Huntingtin siRNA
aagaggaggaggccgacgccc

SEQ ID NO: 56 - DNA, 19 bp, Artificial
  nonsense siRNA
aguacugcuuacgauacgg

SEQ ID NO: 57 - DNA, 19 bp, Artificial
  nonsense siRNA
ccguaucguaagcaguacu

SEQ ID NO: 58 - DNA, 19 bp, Artificial
  nNOS-specific siRNA
caaagagatcgacaccatc

SEQ ID NO: 59 - DNA, 21 bp, Artificial
  nNOS specific siRNA
gatggtgtcgatctctttgtt

SEQ ID NO: 60 - DNA, 19 bp, Artificial
  nNOS-specific siRNA
cacgcatgtctggaaaggc

SEQ ID NO: 61 - DNA, 21 bp, Artificial
  nNOS-specific siRNA
gcctttccagacatgcgtgtt

SEQ ID NO: 62 - DNA, 19 bp, Artificial
  nNOS - specific siRNA
ggtctatccaatgtccaca

SEQ ID NO: 63 - DNA, 21 bp, Artificial
  nNOS-specific siRNA
tgtggacattggatagacctt

SEQ ID NO: 64 - DNA, 19 bp, Artificial
  iNOS-specific siRNA
ccaccagtatgcaatgaat

SEQ ID NO: 65 - DNA, 21 bp, Artificial
  iNOS-specific siRNA
acaacaggaaccuaccagctt

SEQ ID NO: 66 - DNA, 21 bp, Artificial
  iNOS-specific siRNA
gcugguagguuccuguugutt

SEQ ID NO: 67 - DNA, 21 bp, Artificial
  iNOS-specific antisense
acagctcagtcccttcaccaa

SEQ ID NO: 68 - DNA, 18 bp, Artificial
  iNOS-specific antisense
tttgccttatactgttcc

SEQ ID NO: 69 - RNA, 19 nt, Artificial
  nonsense siRNA
aguacugcuuacgauacgg

SEQ ID NO: 70 - RNA, 19 nt, Artificial
  nonsense siRNA
ccguaucguaagcaguacu